European Patent Application EP 4 582 435 A1, published July 9, 2025. Title: carrier peptide fragment and use thereof. Applicant: TOAGOSEI CO., LTD. The sequence listing filed with the application follows.

SEQUENCE LISTING (15 sequences)

SEQ ID NO: 1 - protein, 13 aa, synthetic construct
  SITE 12: note = D-Lysine
KKRTLRKSNRKKR

SEQ ID NO: 2 - protein, 13 aa, synthetic construct
KKRTLRKSNRKKR

SEQ ID NO: 3 - protein, 13 aa, synthetic construct
  SITE 1: note = D-Lysine
KKRTLRKSNRKKR

SEQ ID NO: 4 - protein, 13 aa, synthetic construct
  SITE 2: note = D-Lysine
KKRTLRKSNRKKR

SEQ ID NO: 5 - protein, 13 aa, synthetic construct
  SITE 3: note = D-Arginine
KKRTLRKSNRKKR

SEQ ID NO: 6 - protein, 13 aa, synthetic construct
  SITE 4: note = D-Threonine
KKRTLRKSNRKKR

SEQ ID NO: 7 - protein, 13 aa, synthetic construct
  SITE 5: note = D-Leucine
KKRTLRKSNRKKR

SEQ ID NO: 8 - protein, 13 aa, synthetic construct
  SITE 6: note = D-Arginine
KKRTLRKSNRKKR

SEQ ID NO: 9 - protein, 13 aa, synthetic construct
  SITE 7: note = D-Lysine
KKRTLRKSNRKKR

SEQ ID NO: 10 - protein, 13 aa, synthetic construct
  SITE 8: note = D-Serine
KKRTLRKSNRKKR

SEQ ID NO: 11 - protein, 13 aa, synthetic construct
  SITE 9: note = D-Asparagine
KKRTLRKSNRKKR

SEQ ID NO: 12 - protein, 13 aa, synthetic construct
  SITE 10: note = D-Arginine
KKRTLRKSNRKKR

SEQ ID NO: 13 - protein, 13 aa, synthetic construct
  SITE 11: note = D-Lysine
KKRTLRKSNRKKR

SEQ ID NO: 14 - protein, 13 aa, synthetic construct
  SITE 13: note = D-Arginine
KKRTLRKSNRKKR

SEQ ID NO: 15 - protein, 13 aa, synthetic construct
  SITE 1: note = D-Lysine
  SITE 2: note = D-Lysine
  SITE 3: note = D-Arginine
  SITE 4: note = D-Threonine
  SITE 5: note = D-Leucine
  SITE 6: note = D-Arginine
  SITE 7: note = D-Lysine
  SITE 8: note = D-Serine
  SITE 9: note = D-Asparagine
  SITE 10: note = D-Arginine
  SITE 11: note = D-Lysine
  SITE 12: note = D-Lysine
  SITE 13: note = D-Arginine
KKRTLRKSNRKKR